European Patent Specification EP 4 043 490 B1, published August 27, 2025. Title: HUMANIZED ANTI-VEGF ANTIBODY FAB FRAGMENT AND USE THEREOF. Applicant: SinoCellTech Ltd. The sequence listing filed with the application follows.

SEQUENCE LISTING (55 sequences)

SEQ ID NO: 1 - protein, 191 aa, Artificial Sequence
  Amino acid sequence of Met 1- Arg191 of the human VEGF protein (UniProtKB P15692)
MNFLLSWVHWSLALLLYLHHAKWSQAAPMAEGGGQNHHEVVKFMDVYQRSYCHPIETLVDIFQEYPDEIEYIFKPSCVPLMRCGGCCNDEGLECVPTEESNITMQIMRIKPHQGQHIGEMSFLQHNKCECRPKKDRARQEKKSVRGKGKGQKRKRKKSRYKSWSVYVGARCCLMPWSLPGPHPCGPCSERR

SEQ ID NO: 2 - DNA, 54 bp, Artificial Sequence
  Nucleotide sequence of the linker used in the construction of the phage antibody library for the linkage of the rabbit antibody scFv
tctagtggtggcggtggttcgggcggtggtggaggtggtagttctagatcttcc

SEQ ID NO: 3 - DNA, 738 bp, Artificial Sequence
  Nucleotide sequence of the rabbit antibody scFv used in the construction of antibody VEGF165-R988
gagctcgatctgacccagactccatcccccgtgtctgcggctgttggaggcacagtcaccatcaattgccagtccagtcagactatttatgctaacaggcgcttagcctggtatcaacagaaaccagggcagcctcccaagctcctgatctatggtgcatccactctggcatctggggtcccatcgcggttcaaaggcagtggatctgggacacagttcactctcaccatcagcggcgtgcagtgtgacgatgctgccacttactactgtgcaggctataaaagttatgatggtgatgatgttggtttcggcggagggaccgaggtggtcgtcaaatctagtggtggcggtggttcgggcggtggtggaggtggtagttctagatcttcccagtcggtggaggagtccgggggtcgcctggtaacgcctgggacacccctgacactcacctgcacagtctctggaatcgacctcagtagctatgcaataagctgggtccgccaggctccagggaaggggctggaatacatcggatacatttggaatgctggtaacacctactacgcgagctgggcaaaaggccgattcaccatctccaaaacctcgaccacggtggatctgaaaatcaccagtccgacaaccgaggacacggccacctatttctgtgccagaggaacattaggggactacaatggcatggacccctggggcccagggaccctcgtcaccgtctcttca

SEQ ID NO: 4 - DNA, 348 bp, Artificial Sequence
  Nucleotide sequence of the heavy chain variable region of rabbit antibody VEGF165-R988
cagtcggtggaggagtccgggggtcgcctggtaacgcctgggacacccctgacactcacctgcacagtctctggaatcgacctcagtagctatgcaataagctgggtccgccaggctccagggaaggggctggaatacatcggatacatttggaatgctggtaacacctactacgcgagctgggcaaaaggccgattcaccatctccaaaacctcgaccacggtggatctgaaaatcaccagtccgacaaccgaggacacggccacctatttctgtgccagaggaacattaggggactacaatggcatggacccctggggcccagggaccctcgtcaccgtctcttca

SEQ ID NO: 5 - DNA, 336 bp, Artificial Sequence
  Nucleotide sequence of the light chain variable region of rabbit antibody VEGF165-R988
gagctcgatctgacccagactccatcccccgtgtctgcggctgttggaggcacagtcaccatcaattgccagtccagtcagactatttatgctaacaggcgcttagcctggtatcaacagaaaccagggcagcctcccaagctcctgatctatggtgcatccactctggcatctggggtcccatcgcggttcaaaggcagtggatctgggacacagttcactctcaccatcagcggcgtgcagtgtgacgatgctgccacttactactgtgcaggctataaaagttatgatggtgatgatgttggtttcggcggagggaccgaggtggtcgtcaaa

SEQ ID NO: 6 - DNA, 972 bp, Artificial Sequence
  Nucleotide sequence of the heavy chain constant region of rabbit IgG1
ggtcaacctaaggctccgtcagtcttcccactggccccctgctgcggggacacacccagctccacggtgaccctgggctgcctggtcaaaggctacctcccggagccagtgaccgtgacctggaactcgggcaccctcaccaatggggtacgcaccttcccgtccgtccggcagtcctcaggcctctactcgctgagcagcgtggtgagcgtgacctcaagcagccagcccgtcacctgcaacgtggcccacccagccaccaacaccaaagtggacaagaccgttgcgccctcgacatgcagcaagcccacgtgcccaccccctgaactcctggggggaccgtctgtcttcatcttccccccaaaacccaaggacaccctcatgatctcacgcacccccgaggtcacatgcgtggtggtggacgtgagccaggatgaccccgaggtgcagttcacatggtacataaacaacgagcaggtgcgcaccgcccggccgccgctacgggagcagcagttcaacagcacgatccgcgtggtcagcaccctccccatcgcgcaccaggactggctgaggggcaaggagttcaagtgcaaagtccacaacaaggcactcccggcccccatcgagaaaaccatctccaaagccagagggcagcccctggagccgaaggtctacaccatgggccctccccgggaggagctgagcagcaggtcggtcagcctgacctgcatgatcaacggcttctacccttccgacatctcggtggagtgggagaagaacgggaaggcagaggacaactacaagaccacgccggccgtgctggacagcgacggctcctacttcctctacagcaagctctcagtgcccacgagtgagtggcagcggggcgacgtcttcacctgctccgtgatgcacgaggccttgcacaaccactacacgcagaagtccatctcccgctctccgggtaaataa

SEQ ID NO: 7 - DNA, 315 bp, Artificial Sequence
  Nucleotide sequence of the constant region of rabbit kappa light chain
ggggatccagttgcacctactgtcctcatcttcccaccagctgctgatcaggtggcaactggaacagtcaccatcgtgtgtgtggcgaataaatactttcccgatgtcaccgtcacctgggaggtggatggcaccacccaaacaactggcatcgagaacagtaaaacaccgcagaattctgcagattgtacctacaacctcagcagcactctgacactgaccagcacacagtacaacagccacaaagagtacacctgcaaggtgacccagggcacgacctcagtcgtccagagcttcaataggggtgactgttaa

SEQ ID NO: 8 - protein, 116 aa, Artificial Sequence
  Amino acid sequence of the heavy chain variable region of rabbit antibody VEGF165-R988
QSVEESGGRLVTPGTPLTLTCTVSGIDLSSYAISWVRQAPGKGLEYIGYIWNAGNTYYASWAKGRFTISKTSTTVDLKITSPTTEDTATYFCARGTLGDYNGMDPWGPGTLVTVSS

SEQ ID NO: 9 - protein, 112 aa, Artificial Sequence
  Amino acid sequence of the light chain variable region of rabbit antibody VEGF165-R988
ELDLTQTPSPVSAAVGGTVTINCQSSQTIYANRRLAWYQQKPGQPPKLLIYGASTLASGVPSRFKGSGSGTQFTLTISGVQCDDAATYYCAGYKSYDGDDVGFGGGTEVVVK

SEQ ID NO: 10 - protein, 13 aa, Artificial Sequence
  Amino acid sequence of the light chain CDR1 of rabbit antibody VEGF165-R988
QSSQTIYANRRLA

SEQ ID NO: 11 - protein, 7 aa, Artificial Sequence
  Amino acid sequence of the light chain CDR2 of rabbit antibody VEGF165-R988
GASTLAS

SEQ ID NO: 12 - protein, 12 aa, Artificial Sequence
  Amino acid sequence of the light chain CDR3 of rabbit antibody VEGF165-R988
AGYKSYDGDDVG

SEQ ID NO: 13 - protein, 10 aa, Artificial Sequence
  Amino acid sequence of the heavy chain CDR1 of rabbit antibody VEGF165-R988
GIDLSSYAIS

SEQ ID NO: 14 - protein, 16 aa, Artificial Sequence
  Amino acid sequence of the heavy chain CDR2 of rabbit antibody VEGF165-R988
YIWNAGNTYYASWAKG

SEQ ID NO: 15 - protein, 13 aa, Artificial Sequence
  Amino acid sequence of the heavy chain CDR3 of rabbit antibody VEGF165-R988
ARGTLGDYNGMDP

SEQ ID NO: 16 - DNA, 1404 bp, Artificial Sequence
  Nucleotide sequence of the humanized antibody VEGF165-H988-10 heavy chain containing signal peptide
atgggctggtccctgattctgctgttcctggtggctgtggctaccagggtgctgagtcagtctgtccaggagtctggacctggactggtgaagccatctgagaccctgtccctgacttgtactgtgtctggcattgacctgtcctcctatgccatctcctgggtgagacaacctcctggcaagggattggaatacattggctacatctggaatgctggcaacacctactatgcctcctgggctaagggcagggtgaccatctctgtggacaccagcaagaaccaggtggacctgaaactgtcctctgtgacagcagcagacacagcagtctacttctgtgccaggggcaccctgggagactacaatgggatggacccatggggacctggcaccctggtgacagtgtccagcgctagcaccaagggcccatcggtcttccccctggcaccctcctccaagagcacctctgggggcacagcggccctgggctgcctggtcaaggactacttccccgaaccggtgacggtgtcgtggaactcaggcgccctgaccagcggcgtgcacaccttcccggctgtcctacagtcctcaggactctactccctcagcagcgtggtgaccgtgccctccagcagcttgggcacccagacctacatctgcaacgtgaatcacaagcccagcaacaccaaggtggacaagaaagttgagcccaaatcttgtgacaaaactcacacatgcccaccgtgcccagcacctgaactcctggggggaccgtcagtcttcctcttccccccaaaacccaaggacaccctcatgatctcccggacccctgaggtcacgtgcgtggtggtggacgtgagccacgaagaccccgaggtcaagttcaactggtacgtggacggcgtggaggtgcataatgccaagacaaagccgcgggaggagcagtacaacagcacgtaccgtgtggtcagcgtcctcaccgtcctgcaccaggactggctgaatggcaaggagtacaagtgcaaggtctccaacaaagccctcccagcccccatcgagaaaaccatctccaaagccaaagggcagccccgagaaccacaggtgtacaccctgcccccatcccgggatgagctgaccaagaaccaggtcagcctgacctgcctggtcaaaggcttctatcccagcgacatcgccgtggagtgggagagcaatgggcagccggagaacaactacaagaccacgcctcccgtgctggactccgacggctccttcttcctctacagcaagctcaccgtggacaagagcaggtggcagcaggggaacgtcttctcatgctccgtgatgcatgaggctctgcacaaccactacacgcagaagagcctctccctgtctccgggtaaatga

SEQ ID NO: 17 - DNA, 717 bp, Artificial Sequence
  Nucleotide sequence of the humanized antibody VEGF165-H988-10 light chain containing signal peptide
atgggctggtcctgtatcatcctgttcctggtggctacagccacaggagtgcatagtgaactccaacttacccagagcccatcctccctgtctgcctctgtgggagacagggtgaccatcacttgtcagtccagccagaccatctatgccaacaggagactggcttggtatcaacagaagcctggcaaggtgccaaaactgctgatttatggagccagcaccctggcatctggagtgccaagcaggttcaagggctctggctctggcacagacttcaccctgaccatctcctccctccaacctgaggatgtggctacctactactgtgctggctacaagtcctatgatggagatgatgtgggctttggaggaggcaccaaggtggagattaagcgtacggtggctgcaccatctgtcttcatcttcccgccatctgatgagcagttgaaatctggaactgcctctgttgtgtgcctgctgaataacttctatcccagagaggccaaagtacagtggaaggtggataacgccctccaatcgggtaactcccaggagagtgtcacagagcaggacagcaaggacagcacctacagcctcagcagcaccctgacgctgagcaaagcagactacgagaaacacaaagtctacgcctgcgaagtcacccatcagggcctgagctcgcccgtcacaaagagcttcaacaggggagagtgttag

SEQ ID NO: 18 - protein, 467 aa, Artificial Sequence
  Amino acid sequence of the heavy chain of humanized antibody VEGF165-H988-10 containing signal peptide
MGWSLILLFLVAVATRVLSQSVQESGPGLVKPSETLSLTCTVSGIDLSSYAISWVRQPPGKGLEYIGYIWNAGNTYYASWAKGRVTISVDTSKNQVDLKLSSVTAADTAVYFCARGTLGDYNGMDPWGPGTLVTVSSASTKGPSVFPLAPSSKSTSGGTAALGCLVKDYFPEPVTVSWNSGALTSGVHTFPAVLQSSGLYSLSSVVTVPSSSLGTQTYICNVNHKPSNTKVDKKVEPKSCDKTHTCPPCPAPELLGGPSVFLFPPKPKDTLMISRTPEVTCVVVDVSHEDPEVKFNWYVDGVEVHNAKTKPREEQYNSTYRVVSVLTVLHQDWLNGKEYKCKVSNKALPAPIEKTISKAKGQPREPQVYTLPPSRDELTKNQVSLTCLVKGFYPSDIAVEWESNGQPENNYKTTPPVLDSDGSFFLYSKLTVDKSRWQQGNVFSCSVMHEALHNHYTQKSLSLSPGK

SEQ ID NO: 19 - protein, 238 aa, Artificial Sequence
  Amino acid sequence of the light chain of humanized antibody VEGF165-H988-10 containing signal peptide
MGWSCIILFLVATATGVHSELQLTQSPSSLSASVGDRVTITCQSSQTIYANRRLAWYQQKPGKVPKLLIYGASTLASGVPSRFKGSGSGTDFTLTISSLQPEDVATYYCAGYKSYDGDDVGFGGGTKVEIKRTVAAPSVFIFPPSDEQLKSGTASVVCLLNNFYPREAKVQWKVDNALQSGNSQESVTEQDSKDSTYSLSSTLTLSKADYEKHKVYACEVTHQGLSSPVTKSFNRGEC

SEQ ID NO: 20 - DNA, 354 bp, Artificial Sequence
  Nucleotide sequence of the heavy chain variable region of humanized antibody VEGF165-H988-10
cagtctgtccaggagtctggacctggactggtgaagccatctgagaccctgtccctgacttgtactgtgtctggcattgacctgtcctcctatgccatctcctgggtgagacaacctcctggcaagggattggaatacattggctacatctggaatgctggcaacacctactatgcctcctgggctaagggcagggtgaccatctctgtggacaccagcaagaaccaggtggacctgaaactgtcctctgtgacagcagcagacacagcagtctacttctgtgccaggggcaccctgggagactacaatgggatggacccatggggacctggcaccctggtgacagtgtccagc

SEQ ID NO: 21 - DNA, 336 bp, Artificial Sequence
  Nucleotide sequence of the light chain variable region of humanized antibody VEGF165-H988-10
gaactccaacttacccagagcccatcctccctgtctgcctctgtgggagacagggtgaccatcacttgtcagtccagccagaccatctatgccaacaggagactggcttggtatcaacagaagcctggcaaggtgccaaaactgctgatttatggagccagcaccctggcatctggagtgccaagcaggttcaagggctctggctctggcacagacttcaccctgaccatctcctccctccaacctgaggatgtggctacctactactgtgctggctacaagtcctatgatggagatgatgtgggctttggaggaggcaccaaggtggagattaag

SEQ ID NO: 22 - protein, 118 aa, Artificial Sequence
  Amino acid sequence of the heavy chain variable region of antibody VEGF165-H988-10
QSVQESGPGLVKPSETLSLTCTVSGIDLSSYAISWVRQPPGKGLEYIGYIWNAGNTYYASWAKGRVTISVDTSKNQVDLKLSSVTAADTAVYFCARGTLGDYNGMDPWGPGTLVTVSS

SEQ ID NO: 23 - protein, 112 aa, Artificial Sequence
  Amino acid sequence of the light chain variable region of antibody VEGF165-H988-10
ELQLTQSPSSLSASVGDRVTITCQSSQTIYANRRLAWYQQKPGKVPKLLIYGASTLASGVPSRFKGSGSGTDFTLTISSLQPEDVATYYCAGYKSYDGDDVGFGGGTKVEIK

SEQ ID NO: 24 - protein, 13 aa, Artificial Sequence
  Amino acid sequence of the light chain CDR1 of humanized antibody VEGF-H988 Fab fragment
QSSKFLWQGRRLA

SEQ ID NO: 25 - protein, 7 aa, Artificial Sequence
  Amino acid sequence of the light chain CDR2 of humanized antibody VEGF-H988 Fab fragment
GASTLAS

SEQ ID NO: 26 - protein, 12 aa, Artificial Sequence
  Amino acid sequence of the light chain CDR3 of humanized antibody VEGF-H988 Fab fragment
AGYKSYDGDVVG

SEQ ID NO: 27 - protein, 10 aa, Artificial Sequence
  Amino acid sequence of the heavy chain CDR1 of humanized antibody VEGF-H988 Fab fragment
GIDLSSYAIS

SEQ ID NO: 28 - protein, 16 aa, Artificial Sequence
  Amino acid sequence of the heavy chain CDR2 of humanized antibody VEGF-H988 Fab fragment
YIWNDLFTYYASWAKG

SEQ ID NO: 29 - protein, 13 aa, Artificial Sequence
  Amino acid sequence of the heavy chain CDR3 of humanized antibody VEGF-H988 Fab fragment
ARGTLGDYGGMDP

SEQ ID NO: 30 - protein, 221 aa, Artificial Sequence
  Amino acid sequence of the heavy chain of humanized antibody VEGF-H988 Fab fragment
QSVQESGPGLVKPSETLSLTCTVSGIDLSSYAISWVRQPPGKGLEYIGYIWNDLFTYYASWAKGRVTISVDTSKNQVDLKLSSVTAADTAVYFCARGTLGDYGGMDPWGQGTLVTVSSASTKGPSVFPLAPSSKSTSGGTAALGCLVKDYFPEPVTVSWNSGALTSGVHTFPAVLQSSGLYSLSSVVTVPSSSLGTQTYICNVNHKPSNTKVDKKVEPKSC

SEQ ID NO: 31 - protein, 219 aa, Artificial Sequence
  Amino acid sequence of the light chain of humanized antibody VEGF-H988 Fab fragment
ELQLTQSPSSLSASVGDRVTITCQSSKFLWQGRRLAWYQQKPGKVPKLLIYGASTLASGVPSRFKGSGSGTDFTLTISSLQPEDVATYYCAGYKSYDGDVVGFGGGTKVEIKRTVAAPSVFIFPPSDEQLKSGTASVVCLLNNFYPREAKVQWKVDNALQSGNSQESVTEQDSKDSTYSLSSTLTLSKADYEKHKVYACEVTHQGLSSPVTKSFNRGEC

SEQ ID NO: 32 - protein, 240 aa, Artificial Sequence
  Amino acid sequence of the heavy chain of humanized antibody VEGF-H988 Fab fragment containing signal peptide
MGWSLILLFLVAVATRVLSQSVQESGPGLVKPSETLSLTCTVSGIDLSSYAISWVRQPPGKGLEYIGYIWNDLFTYYASWAKGRVTISVDTSKNQVDLKLSSVTAADTAVYFCARGTLGDYGGMDPWGQGTLVTVSSASTKGPSVFPLAPSSKSTSGGTAALGCLVKDYFPEPVTVSWNSGALTSGVHTFPAVLQSSGLYSLSSVVTVPSSSLGTQTYICNVNHKPSNTKVDKKVEPKSC

SEQ ID NO: 33 - protein, 238 aa, Artificial Sequence
  Amino acid sequence of the light chain of humanized antibody VEGF-H988 Fab fragment containing signal peptide
MGWSCIILFLVATATGVHSELQLTQSPSSLSASVGDRVTITCQSSKFLWQGRRLAWYQQKPGKVPKLLIYGASTLASGVPSRFKGSGSGTDFTLTISSLQPEDVATYYCAGYKSYDGDVVGFGGGTKVEIKRTVAAPSVFIFPPSDEQLKSGTASVVCLLNNFYPREAKVQWKVDNALQSGNSQESVTEQDSKDSTYSLSSTLTLSKADYEKHKVYACEVTHQGLSSPVTKSFNRGEC

SEQ ID NO: 34 - protein, 19 aa, Artificial Sequence
  Amino acid sequence of heavy chain signal peptide
MGWSLILLFLVAVATRVLS

SEQ ID NO: 35 - protein, 19 aa, Artificial Sequence
  Amino acid sequence of light chain signal peptide
MGWSCIILFLVATATGVHS

SEQ ID NO: 36 - protein, 118 aa, Artificial Sequence
  Amino acid sequence of the heavy chain variable region of humanized antibody VEGF-H988 Fab fragment
QSVQESGPGLVKPSETLSLTCTVSGIDLSSYAISWVRQPPGKGLEYIGYIWNDLFTYYASWAKGRVTISVDTSKNQVDLKLSSVTAADTAVYFCARGTLGDYGGMDPWGQGTLVTVSS

SEQ ID NO: 37 - protein, 112 aa, Artificial Sequence
  Amino acid sequence of the light chain variable region of humanized antibody VEGF-H988 Fab fragment
ELQLTQSPSSLSASVGDRVTITCQSSKFLWQGRRLAWYQQKPGKVPKLLIYGASTLASGVPSRFKGSGSGTDFTLTISSLQPEDVATYYCAGYKSYDGDVVGFGGGTKVEIK

SEQ ID NO: 38 - protein, 330 aa, Artificial Sequence [sequence omitted]

SEQ ID NO: 39 - protein, 107 aa, Artificial Sequence [sequence omitted]

SEQ ID NO: 40 - protein, 103 aa, Artificial Sequence
  Amino acid sequence of human IgG1  heavy chain CH1 constant region
ASTKGPSVFPLAPSSKSTSGGTAALGCLVKDYFPEPVTVSWNSGALTSGVHTFPAVLQSSGLYSLSSVVTVPSSSLGTQTYICNVNHKPSNTKVDKKVEPKSC

SEQ ID NO: 41 - DNA, 723 bp, Artificial Sequence
  Nucleotide sequence of humanized antibody VEGF-H988 Fab fragment heavy chain containing signal peptide
atgggctggtccctgattctgctgttcctggtggctgtggctaccagggtgctgagtcagtctgtccaggagtctggacctggactggtgaagccatctgagaccctgtccctgacttgtactgtgtctggcattgacctgtcctcctatgccatctcctgggtgagacaacctcctggcaagggattggaatacattggctacatctggaatgatctcttcacctactatgcctcctgggctaagggcagggtgaccatctctgtggacaccagcaagaaccaggtggacctgaaactgtcctctgtgacagcagcagacacagcagtctacttctgtgccaggggcaccctgggagactacggcgggatggacccatggggacagggcaccctggtgacagtgtccagcgcaagcaccaagggcccatcggtcttccccctggcaccctcctccaagagcacctctgggggcacagcggccctgggctgcctggtcaaggactacttccccgaaccggtgacggtgtcgtggaactcaggcgccctgaccagcggcgtgcacaccttcccggctgtcctacagtcctcaggactctactccctcagcagcgtggtgaccgtgccctccagcagcttgggcacccagacctacatctgcaacgtgaatcacaagcccagcaacaccaaggtggacaagaaagttgagcccaaatcttgttaa

SEQ ID NO: 42 - DNA, 717 bp, Artificial Sequence
  Nucleotide sequence of humanized antibody VEGF-H988 Fab fragment light chain containing signal peptide
atgggctggtcctgtatcatcctgttcctggtggctacagccacaggagtgcatagtgaactccaacttacccagagcccatcctccctgtctgcctctgtgggagacagggtgaccatcacttgtcagtccagcaagttcctctggcagggcaggagactggcttggtatcaacagaagcctggcaaggtgccaaaactgctgatttatggagccagcaccctggcatctggagtgccaagcaggttcaagggctctggctctggcacagacttcaccctgaccatctcctccctccaacctgaggatgtggctacctactactgtgctggctacaagtcctatgatggagatgttgtgggctttggaggaggcaccaaggtggagattaagcgtacggtggctgcaccatctgtcttcatcttcccgccatctgatgagcagttgaaatctggaactgcctctgttgtgtgcctgctgaataacttctatcccagagaggccaaagtacagtggaaggtggataacgccctccaatcgggtaactcccaggagagtgtcacagagcaggacagcaaggacagcacctacagcctcagcagcaccctgacgctgagcaaagcagactacgagaaacacaaagtctacgcctgcgaagtcacccatcagggcctgagctcgcccgtcacaaagagcttcaacaggggagagtgttaa

SEQ ID NO: 43 - DNA, 57 bp, Artificial Sequence
  Nucleotide sequence of heavy chain signal peptide
atgggctggtccctgattctgctgttcctggtggctgtggctaccagggtgctgagt

SEQ ID NO: 44 - DNA, 57 bp, Artificial Sequence
  Nucleotide sequence of light chain signal peptide
atgggctggtcctgtatcatcctgttcctggtggctacagccacaggagtgcatagt

SEQ ID NO: 45 - DNA, 354 bp, Artificial Sequence
  Nucleotide sequence of the heavy chain variable region of humanized antibody VEGF-H988 Fab fragment
cagtctgtccaggagtctggacctggactggtgaagccatctgagaccctgtccctgacttgtactgtgtctggcattgacctgtcctcctatgccatctcctgggtgagacaacctcctggcaagggattggaatacattggctacatctggaatgatctcttcacctactatgcctcctgggctaagggcagggtgaccatctctgtggacaccagcaagaaccaggtggacctgaaactgtcctctgtgacagcagcagacacagcagtctacttctgtgccaggggcaccctgggagactacggcgggatggacccatggggacagggcaccctggtgacagtgtccagc

SEQ ID NO: 46 - DNA, 336 bp, Artificial Sequence
  Nucleotide sequence of the light chain variable region of humanized antibody VEGF-H988 Fab fragment
gaactccaacttacccagagcccatcctccctgtctgcctctgtgggagacagggtgaccatcacttgtcagtccagcaagttcctctggcagggcaggagactggcttggtatcaacagaagcctggcaaggtgccaaaactgctgatttatggagccagcaccctggcatctggagtgccaagcaggttcaagggctctggctctggcacagacttcaccctgaccatctcctccctccaacctgaggatgtggctacctactactgtgctggctacaagtcctatgatggagatgttgtgggctttggaggaggcaccaaggtggagattaag

SEQ ID NO: 47 - DNA, 993 bp, Artificial Sequence
  Nucleotide sequence of human IgG1 heavy chain constant region
gcaagcaccaagggcccatcggtcttccccctggcaccctcctccaagagcacctctgggggcacagcggccctgggctgcctggtcaaggactacttccccgaaccggtgacggtgtcgtggaactcaggcgccctgaccagcggcgtgcacaccttcccggctgtcctacagtcctcaggactctactccctcagcagcgtggtgaccgtgccctccagcagcttgggcacccagacctacatctgcaacgtgaatcacaagcccagcaacaccaaggtggacaagaaagttgagcccaaatcttgtgacaaaactcacacatgcccaccgtgcccagcacctgaactcctggggggaccgtcagtcttcctcttccccccaaaacccaaggacaccctcatgatctcccggacccctgaggtcacgtgcgtggtggtggacgtgagccacgaagaccccgaggtcaagttcaactggtacgtggacggcgtggaggtgcataatgccaagacaaagccgcgggaggagcagtacaacagcacgtaccgtgtggtcagcgtcctcaccgtcctgcaccaggactggctgaatggcaaggagtacaagtgcaaggtctccaacaaagccctcccagcccccatcgagaaaaccatctccaaagccaaagggcagccccgagaaccacaggtgtacaccctgcccccatcccgggatgagctgaccaagaaccaggtcagcctgacctgcctggtcaaaggcttctatcccagcgacatcgccgtggagtgggagagcaatgggcagccggagaacaactacaagaccacgcctcccgtgctggactccgacggctccttcttcctctacagcaagctcaccgtggacaagagcaggtggcagcaggggaacgtcttctcatgctccgtgatgcatgaggctctgcacaaccactacacgcagaagagcctctccctgtctccgggtaaataa

SEQ ID NO: 48 - DNA, 324 bp, Artificial Sequence
  Nucleotide sequence of human kappa light chain constant region
cgtacggtggctgcaccatctgtcttcatcttcccgccatctgatgagcagttgaaatctggaactgcctctgttgtgtgcctgctgaataacttctatcccagagaggccaaagtacagtggaaggtggataacgccctccaatcgggtaactcccaggagagtgtcacagagcaggacagcaaggacagcacctacagcctcagcagcaccctgacgctgagcaaagcagactacgagaaacacaaagtctacgcctgcgaagtcacccatcagggcctgagctcgcccgtcacaaagagcttcaacaggggagagtgttaa

SEQ ID NO: 49 - DNA, 312 bp, Artificial Sequence
  Nucleotide sequence of human IgG1 heavy chain CH1 constant region
gcaagcaccaagggcccatcggtcttccccctggcaccctcctccaagagcacctctgggggcacagcggccctgggctgcctggtcaaggactacttccccgaaccggtgacggtgtcgtggaactcaggcgccctgaccagcggcgtgcacaccttcccggctgtcctacagtcctcaggactctactccctcagcagcgtggtgaccgtgccctccagcagcttgggcacccagacctacatctgcaacgtgaatcacaagcccagcaacaccaaggtggacaagaaagttgagcccaaatcttgttaa

SEQ ID NO: 50 - protein, 246 aa, Artificial Sequence
  Amino acid sequence of the rabbit antibody scFv used in the construction of antibody VEGF165-R988
ELDLTQTPSPVSAAVGGTVTINCQSSQTIYANRRLAWYQQKPGQPPKLLIYGASTLASGVPSRFKGSGSGTQFTLTISGVQCDDAATYYCAGYKSYDGDDVGFGGGTEVVVKSSGGGGSGGGGGGSSRSSQSVEESGGRLVTPGTPLTLTCTVSGIDLSSYAISWVRQAPGKGLEYIGYIWNAGNTYYASWAKGRFTISKTSTTVDLKITSPTTEDTATYFCARGTLGDYNGMDPWGPGTLVTVSS

SEQ ID NO: 51 - protein, 18 aa, Artificial Sequence
  Amino acid sequence of the linker used in the construction of the phage antibody library for the linkage of rabbit antibody scFv
SSGGGGSGGGGGGSSRSS

SEQ ID NO: 52 - DNA, 1377 bp, Artificial Sequence
  Nucleotide sequence of the rabbit antibody VEGF165-R988 heavy chain containing signal peptide
atgggctggtccctgattctgctgttcctggtggctgtggctaccagggtgctgagtcagtcggtggaggagtccgggggtcgcctggtaacgcctgggacacccctgacactcacctgcacagtctctggaatcgacctcagtagctatgcaataagctgggtccgccaggctccagggaaggggctggaatacatcggatacatttggaatgctggtaacacctactacgcgagctgggcaaaaggccgattcaccatctccaaaacctcgaccacggtggatctgaaaatcaccagtccgacaaccgaggacacggccacctatttctgtgccagaggaacattaggggactacaatggcatggacccctggggcccagggaccctcgtcaccgtctcttcaggtcaacctaaggctccgtcagtcttcccactggccccctgctgcggggacacacccagctccacggtgaccctgggctgcctggtcaaaggctacctcccggagccagtgaccgtgacctggaactcgggcaccctcaccaatggggtacgcaccttcccgtccgtccggcagtcctcaggcctctactcgctgagcagcgtggtgagcgtgacctcaagcagccagcccgtcacctgcaacgtggcccacccagccaccaacaccaaagtggacaagaccgttgcgccctcgacatgcagcaagcccacgtgcccaccccctgaactcctggggggaccgtctgtcttcatcttccccccaaaacccaaggacaccctcatgatctcacgcacccccgaggtcacatgcgtggtggtggacgtgagccaggatgaccccgaggtgcagttcacatggtacataaacaacgagcaggtgcgcaccgcccggccgccgctacgggagcagcagttcaacagcacgatccgcgtggtcagcaccctccccatcgcgcaccaggactggctgaggggcaaggagttcaagtgcaaagtccacaacaaggcactcccggcccccatcgagaaaaccatctccaaagccagagggcagcccctggagccgaaggtctacaccatgggccctccccgggaggagctgagcagcaggtcggtcagcctgacctgcatgatcaacggcttctacccttccgacatctcggtggagtgggagaagaacgggaaggcagaggacaactacaagaccacgccggccgtgctggacagcgacggctcctacttcctctacagcaagctctcagtgcccacgagtgagtggcagcggggcgacgtcttcacctgctccgtgatgcacgaggccttgcacaaccactacacgcagaagtccatctcccgctctccgggtaaataa

SEQ ID NO: 53 - DNA, 708 bp, Artificial Sequence
  Nucleotide sequence of the rabbit antibody VEGF165-R988 light chain containing signal peptide
atgggctggtcctgtatcatcctgttcctggtggctacagccacaggagtgcatagtgagctcgatctgacccagactccatcccccgtgtctgcggctgttggaggcacagtcaccatcaattgccagtccagtcagactatttatgctaacaggcgcttagcctggtatcaacagaaaccagggcagcctcccaagctcctgatctatggtgcatccactctggcatctggggtcccatcgcggttcaaaggcagtggatctgggacacagttcactctcaccatcagcggcgtgcagtgtgacgatgctgccacttactactgtgcaggctataaaagttatgatggtgatgatgttggtttcggcggagggaccgaggtggtcgtcaaaggggatccagttgcacctactgtcctcatcttcccaccagctgctgatcaggtggcaactggaacagtcaccatcgtgtgtgtggcgaataaatactttcccgatgtcaccgtcacctgggaggtggatggcaccacccaaacaactggcatcgagaacagtaaaacaccgcagaattctgcagattgtacctacaacctcagcagcactctgacactgaccagcacacagtacaacagccacaaagagtacacctgcaaggtgacccagggcacgacctcagtcgtccagagcttcaataggggtgactgttaa

SEQ ID NO: 54 - protein, 458 aa, Artificial Sequence
  Amino acid sequence of the rabbit antibody VEGF165-R988 heavy chain containing signal peptide
MGWSLILLFLVAVATRVLSQSVEESGGRLVTPGTPLTLTCTVSGIDLSSYAISWVRQAPGKGLEYIGYIWNAGNTYYASWAKGRFTISKTSTTVDLKITSPTTEDTATYFCARGTLGDYNGMDPWGPGTLVTVSSGQPKAPSVFPLAPCCGDTPSSTVTLGCLVKGYLPEPVTVTWNSGTLTNGVRTFPSVRQSSGLYSLSSVVSVTSSSQPVTCNVAHPATNTKVDKTVAPSTCSKPTCPPPELLGGPSVFIFPPKPKDTLMISRTPEVTCVVVDVSQDDPEVQFTWYINNEQVRTARPPLREQQFNSTIRVVSTLPIAHQDWLRGKEFKCKVHNKALPAPIEKTISKARGQPLEPKVYTMGPPREELSSRSVSLTCMINGFYPSDISVEWEKNGKAEDNYKTTPAVLDSDGSYFLYSKLSVPTSEWQRGDVFTCSVMHEALHNHYTQKSISRSPGK

SEQ ID NO: 55 - protein, 235 aa, Artificial Sequence
  Amino acid sequence of the rabbit antibody VEGF165-R988 light chain containing signal peptide
MGWSCIILFLVATATGVHSELDLTQTPSPVSAAVGGTVTINCQSSQTIYANRRLAWYQQKPGQPPKLLIYGASTLASGVPSRFKGSGSGTQFTLTISGVQCDDAATYYCAGYKSYDGDDVGFGGGTEVVVKGDPVAPTVLIFPPAADQVATGTVTIVCVANKYFPDVTVTWEVDGTTQTTGIENSKTPQNSADCTYNLSSTLTLTSTQYNSHKEYTCKVTQGTTSVVQSFNRGDC